European Patent Application EP 4 549 560 A1, published May 7, 2025. Title: ISPETASE-8×CHIMERA RECOMBINASE, ENCODING GENE, RECOMBINANT PLASMID, ENGINEERED STRAIN AND APPLICATIONS. Applicant: Beijing Meihao Biotechnology Co., Ltd. The sequence listing filed with the application follows.

SEQUENCE LISTING (60 sequences)

SEQ ID NO: 1 - protein, 24 aa, IsPETase-1
QTNPYARGPNPTAASLEASAGPFT

SEQ ID NO: 2 - protein, 27 aa, IsPETase-2
VRSFTVSRPSGYGAGTVYYPTNAGGTV

SEQ ID NO: 3 - protein, 28 aa, IsPETase-3
GAIAIVPGYTARQSSIKWWGPRLASHGF

SEQ ID NO: 4 - protein, 53 aa, IsPETase-4
VVITIDTNSTLDQPSSRSSQQMAALRQVASLNGTSSSPIYGKVDTARMGVMGW

SEQ ID NO: 5 - protein, 39 aa, IsPETase-5
SMGGGGSLISAANNPSLKAAAPQAPWDSSTNFSSVTVPT

SEQ ID NO: 6 - protein, 28 aa, IsPETase-6
LIFACENDSIAPVNSSALPIYDSMSRNA

SEQ ID NO: 7 - protein, 39 aa, IsPETase-7
KQFLEINGGSHSCANSGNSNQALIGKKGVAWMKRFMDND

SEQ ID NO: 8 - protein, 25 aa, IsPETase-8
TRYSTFACENPNSTRVSDFRTANCS

SEQ ID NO: 9 - protein, 23 aa, IsPETase-9
ANPYERGPNPTDALLEASSGPFS

SEQ ID NO: 10 - protein, 22 aa, IsPETase-10
SNPYQRGPNPTRSALTADGPFS

SEQ ID NO: 11 - protein, 28 aa, IsPETase-11
VSEENVSRLSASGFGGGTIYYPRENNTY

SEQ ID NO: 12 - protein, 29 aa, IsPETase-12
VATYTVSRLSVSGFGGGVIYYPTGTSLTF

SEQ ID NO: 13 - protein, 28 aa, IsPETase-13
GGIAMSPGYTADASSLAWLGRRLASHGF

SEQ ID NO: 14 - protein, 28 aa, IsPETase-14
GAVAISPGYTGTEASIAWLGERIASHGF

SEQ ID NO: 15 - protein, 50 aa, IsPETase-15
VVITIDTITTLDQPDSRAEQLNAALNHMINRASSTVRSRIDSSRLAVMGH

SEQ ID NO: 16 - protein, 39 aa, IsPETase-16
SMGGGGTLRLASQRPDLKAAIPLTPWHLNKNWSSVTVPT

SEQ ID NO: 17 - protein, 38 aa, IsPETase-17
SMGGGGTLRIAEQNPSLKAAVPLTPWHTDKTFNTSVPV

SEQ ID NO: 18 - protein, 29 aa, IsPETase-18
LIIGADLDTIAPVATHAKPFYNSLPSSIS

SEQ ID NO: 19 - protein, 36 aa, IsPETase-19
KVYVELDNASHFAPNSNNAAISVYTISWMKLWVDND

SEQ ID NO: 20 - protein, 28 aa, IsPETase-20
TRYTQFLCPGPRDGLFGEVEEYRSTCPF

SEQ ID NO: 21 - protein, 289 aa, IsPETase
NFPRASRLMQAAVLGGLMAVSAAATAQTNPYARGPNPTAASLEASAGPFTVRSFTVSRPSGYGAGTVYYPTNAGGTVGAIAIVPGYTARQSSIKWWGPRLASHGFVVITIDTNSTLDQPSSRSSQQMAALRQVASLNGTSSSPIYGKVDTARMGVMGWSMGGGGSLISAANNPSLKAAAPQAPWDSSTNFSSVTVPTLIFACENDSIAPVNSSALPIYDSMSRNAKQFLEINGGSHSCANSGNSNQALIGKKGVAWMKRFMDNDTRYSTFACENPNSTRVSDFRTANCS

SEQ ID NO: 22 - DNA, 783 bp, IsPETase-8*Chimera-1
  source 1..783: mol_type = other DNA
gccaacccctacgagcgcggccccaacccgaccgacgccctgctcgaagccagcagcggccccttctccgtcagcgaggagaacgtctcccggttgagcgccagcggcttcggcggcggcaccatctactacccgcgggagaacaacacctacggcgggatcgccatgtcgccggggtacacggccgacgccagttcgctggcgtggctcgggcggcggttggcatcgcacggcttcgtcgtcatcaccatcgacaccatcaccaccctcgaccagccggacagccgggcagagcagctcaacgccgcgctgaaccacatgatcaaccgggcgtcctccacggtgcgcagccggatcgatagcagccgactggcggtcatgggccactccatgggcggcggcggcaccctgcgtctggcctcccagcgtcccgacctgaaggccgccatcccgctcaccccgtggcacctcaacaagaactggagcagcgtcaccgtgccgacgctgatcatcggggccgacctcgacacgatcgcgccggtcgccacgcacgcgaaaccgttctacaacagcctgccgagctccatcagcaaggtgtacgtggagctcgacaatgcgtcgcacttcgcgcccaacagcaacaacgcggcgatctccgtgtacaccatctcgtggatgaagctgtgggtggataacgacacccgctacacccagttcctctgccccggaccgcgcgacggactcttcggcgaggtcgaagagtaccgctccacctgcccgttc

SEQ ID NO: 23 - DNA, 780 bp, IsPETase-8*Chimera-2
  source 1..780: mol_type = other DNA
gccaacccctacgagcgcggccccaacccgaccgacgccctgctcgaagccagcagcggccccttctccgtcagcgaggagaacgtctcccggttgagcgccagcggcttcggcggcggcaccatctactacccgcgggagaacaacacctacggtgcggtggcgatctcccccggctacaccggcactgaggcttccatcgcctggctgggcgagcgcatcgcctcccacggcttcgtcgtcatcaccatcgacaccatcaccaccctcgaccagccggacagccgggcagagcagctcaacgccgcgctgaaccacatgatcaaccgggcgtcctccacggtgcgcagccggatcgatagcagccgactggcggtcatgggccactccatgggcggcggcggcaccctgcgtctggcctcccagcgtcccgacctgaaggccgccatcccgctcaccccgtggcacctcaacaagaactggagcagcgtcaccgtgccgacgctgatcttcgcctgcgagaacgacagcatcgccccggtcaactcgtccgccctgccgatctacgacagcatgtcgcgcaatgcgaaggtgtacgtggagctcgacaatgcgtcgcacttcgcgcccaacagcaacaacgcggcgatctccgtgtacaccatctcgtggatgaagctgtgggtggataacgacacccgctacacccagttcctctgccccggaccgcgcgacggactcttcggcgaggtcgaagagtaccgctccacctgcccgttc

SEQ ID NO: 24 - DNA, 777 bp, IsPETase-8*Chimera-3
  source 1..777: mol_type = other DNA
tccaacccgtaccagcgcggtcccaaccccacgcggagcgcgctcacggccgacgggccgttctcggtcagcgaggagaacgtctcccggttgagcgccagcggcttcggcggcggcaccatctactacccgcgggagaacaacacctacggtgcggtggcgatctcccccggctacaccggcactgaggcttccatcgcctggctgggcgagcgcatcgcctcccacggcttcgtcgtcatcaccatcgacaccatcaccaccctcgaccagccggacagccgggcagagcagctcaacgccgcgctgaaccacatgatcaaccgggcgtcctccacggtgcgcagccggatcgatagcagccgactggcggtcatgggccactcgatgggcggcggcgggaccctccgcatcgcagagcagaacccgtcgctgaaagcggccgtaccgctcacgccgtggcacaccgacaagacgttcaacacgtcggtaccggtgctgatcatcggggccgacctcgacacgatcgcgccggtcgccacgcacgcgaaaccgttctacaacagcctgccgagctccatcagcaaggtgtacgtggagctcgacaatgcgtcgcacttcgcgcccaacagcaacaacgcggcgatctccgtgtacaccatctcgtggatgaagctgtgggtggataacgacacccgctacacccagttcctctgccccggaccgcgcgacggactcttcggcgaggtcgaagagtaccgctccacctgcccgttc

SEQ ID NO: 25 - DNA, 774 bp, IsPETase-8*Chimera-4
  source 1..774: mol_type = other DNA
gccaacccctacgagcgcggccccaacccgaccgacgccctgctcgaagccagcagcggccccttctccgtggcaacctacaccgtttcgcggctctcggtgagcggcttcgggggcggggtgatctactaccccacaggcacctcgctgaccttcggtgcggtggcgatctcccccggctacaccggcactgaggcttccatcgcctggctgggcgagcgcatcgcctcccacggcttcgtcgtcatcaccatcgacaccatcaccaccctcgaccagccggacagccgggcagagcagctcaacgccgcgctgaaccacatgatcaaccgggcgtcctccacggtgcgcagccggatcgatagcagccgactggcggtcatgggccactcgatgggcggcggcgggaccctccgcatcgcagagcagaacccgtcgctgaaagcggccgtaccgctcacgccgtggcacaccgacaagacgttcaacacgtcggtaccggtgctgatcatcggggccgacctcgacacgatcgcgccggtcgccacgcacgcgaaaccgttctacaacagcctgccgagctccatcagcaaggtgtacgtggagctcgacaatgcgtcgcacttcgcgcccaacagcaacaacgcggcgatctccgtgtacaccatctcgtggatgaagctgtgggtggataacgacacgcgctactccaccttcgcctgcgagaacccgaacagcacccgcgtgtcggacttccgcaccgcgaactgcagc

SEQ ID NO: 26 - DNA, 783 bp, IsPETase-8*Chimera-5
  source 1..783: mol_type = other DNA
gccaacccctacgagcgcggccccaacccgaccgacgccctgctcgaagccagcagcggccccttctccgtggcaacctacaccgtttcgcggctctcggtgagcggcttcgggggcggggtgatctactaccccacaggcacctcgctgaccttcggcgggatcgccatgtcgccggggtacacggccgacgccagttcgctggcgtggctcgggcggcggttggcatcgcacggcttcgtcgtcatcaccatcgacaccatcaccaccctcgaccagccggacagccgggcagagcagctcaacgccgcgctgaaccacatgatcaaccgggcgtcctccacggtgcgcagccggatcgatagcagccgactggcggtcatgggccactcgatgggcggcggcgggaccctccgcatcgcagagcagaacccgtcgctgaaagcggccgtaccgctcacgccgtggcacaccgacaagacgttcaacacgtcggtaccggtgctgatcatcggggccgacctcgacacgatcgcgccggtcgccacgcacgcgaaaccgttctacaacagcctgccgagctccatcagcaaggtgtacgtggagctcgacaatgcgtcgcacttcgcgcccaacagcaacaacgcggcgatctccgtgtacaccatctcgtggatgaagctgtgggtggataacgacacccgctacacccagttcctctgccccggaccgcgcgacggactcttcggcgaggtcgaagagtaccgctccacctgcccgttc

SEQ ID NO: 27 - DNA, 780 bp, IsPETase-8*Chimera-6
  source 1..780: mol_type = other DNA
tccaacccgtaccagcgcggtcccaaccccacgcggagcgcgctcacggccgacgggccgttctcggtggcaacctacaccgtttcgcggctctcggtgagcggcttcgggggcggggtgatctactaccccacaggcacctcgctgaccttcggtgcggtggcgatctcccccggctacaccggcactgaggcttccatcgcctggctgggcgagcgcatcgcctcccacggcttcgtcgtcatcaccatcgacaccatcaccaccctcgaccagccggacagccgggcagagcagctcaacgccgcgctgaaccacatgatcaaccgggcgtcctccacggtgcgcagccggatcgatagcagccgactggcggtcatgggccactccatgggcggcggcggcaccctgcgtctggcctcccagcgtcccgacctgaaggccgccatcccgctcaccccgtggcacctcaacaagaactggagcagcgtcaccgtgccgacgctgatcttcgcctgcgagaacgacagcatcgccccggtcaactcgtccgccctgccgatctacgacagcatgtcgcgcaatgcgaaggtgtacgtggagctcgacaatgcgtcgcacttcgcgcccaacagcaacaacgcggcgatctccgtgtacaccatctcgtggatgaagctgtgggtggataacgacacccgctacacccagttcctctgccccggaccgcgcgacggactcttcggcgaggtcgaagagtaccgctccacctgcccgttc

SEQ ID NO: 28 - DNA, 786 bp, IsPETase-8*Chimera-7
  source 1..786: mol_type = other DNA
cagaccaacccctacgcccgcggcccgaacccgacagccgcctcactcgaagccagcgccggcccgttcaccgtcagcgaggagaacgtctcccggttgagcgccagcggcttcggcggcggcaccatctactacccgcgggagaacaacacctacggtgcggtggcgatctcccccggctacaccggcactgaggcttccatcgcctggctgggcgagcgcatcgcctcccacggcttcgtcgtcatcaccatcgacaccatcaccaccctcgaccagccggacagccgggcagagcagctcaacgccgcgctgaaccacatgatcaaccgggcgtcctccacggtgcgcagccggatcgatagcagccgactggcggtcatgggccactccatgggcggcggcggcaccctgcgtctggcctcccagcgtcccgacctgaaggccgccatcccgctcaccccgtggcacctcaacaagaactggagcagcgtcaccgtgccgacgctgatcatcggggccgacctcgacacgatcgcgccggtcgccacgcacgcgaaaccgttctacaacagcctgccgagctccatcagcaaggtgtacgtggagctcgacaatgcgtcgcacttcgcgcccaacagcaacaacgcggcgatctccgtgtacaccatctcgtggatgaagctgtgggtggataacgacacccgctacacccagttcctctgccccggaccgcgcgacggactcttcggcgaggtcgaagagtaccgctccacctgcccgttc

SEQ ID NO: 29 - DNA, 786 bp, IsPETase-8*Chimera-8
  source 1..786: mol_type = other DNA
cagaccaacccctacgcccgcggcccgaacccgacagccgcctcactcgaagccagcgccggcccgttcaccgtggcaacctacaccgtttcgcggctctcggtgagcggcttcgggggcggggtgatctactaccccacaggcacctcgctgaccttcggtgcggtggcgatctcccccggctacaccggcactgaggcttccatcgcctggctgggcgagcgcatcgcctcccacggcttcgtcgtcatcaccatcgacaccatcaccaccctcgaccagccggacagccgggcagagcagctcaacgccgcgctgaaccacatgatcaaccgggcgtcctccacggtgcgcagccggatcgatagcagccgactggcggtcatgggccactcgatgggcggcggcgggaccctccgcatcgcagagcagaacccgtcgctgaaagcggccgtaccgctcacgccgtggcacaccgacaagacgttcaacacgtcggtaccggtgctgatcatcggggccgacctcgacacgatcgcgccggtcgccacgcacgcgaaaccgttctacaacagcctgccgagctccatcagcaaggtgtacgtggagctcgacaatgcgtcgcacttcgcgcccaacagcaacaacgcggcgatctccgtgtacaccatctcgtggatgaagctgtgggtggataacgacacccgctacacccagttcctctgccccggaccgcgcgacggactcttcggcgaggtcgaagagtaccgctccacctgcccgttc

SEQ ID NO: 30 - DNA, 780 bp, IsPETase-8*Chimera-9
  source 1..780: mol_type = other DNA
gccaacccctacgagcgcggccccaacccgaccgacgccctgctcgaagccagcagcggccccttctccgtggcaacctacaccgtttcgcggctctcggtgagcggcttcgggggcggggtgatctactaccccacaggcacctcgctgaccttcggtgcggtggcgatctcccccggctacaccggcactgaggcttccatcgcctggctgggcgagcgcatcgcctcccacggcttcgtcgtcatcaccatcgacaccatcaccaccctcgaccagccggacagccgggcagagcagctcaacgccgcgctgaaccacatgatcaaccgggcgtcctccacggtgcgcagccggatcgatagcagccgactggcggtcatgggccactcgatgggcggcggcgggaccctccgcatcgcagagcagaacccgtcgctgaaagcggccgtaccgctcacgccgtggcacaccgacaagacgttcaacacgtcggtaccggtgctgatcttcgcctgcgagaacgacagcatcgccccggtcaactcgtccgccctgccgatctacgacagcatgtcgcgcaatgcgaaggtgtacgtggagctcgacaatgcgtcgcacttcgcgcccaacagcaacaacgcggcgatctccgtgtacaccatctcgtggatgaagctgtgggtggataacgacacccgctacacccagttcctctgccccggaccgcgcgacggactcttcggcgaggtcgaagagtaccgctccacctgcccgttc

SEQ ID NO: 31 - DNA, 777 bp, IsPETase-8*Chimera-10
  source 1..777: mol_type = other DNA
gccaacccctacgagcgcggccccaacccgaccgacgccctgctcgaagccagcagcggccccttctccgtggcaacctacaccgtttcgcggctctcggtgagcggcttcgggggcggggtgatctactaccccacaggcacctcgctgaccttcggtgcggtggcgatctcccccggctacaccggcactgaggcttccatcgcctggctgggcgagcgcatcgcctcccacggcttcgtcgtcatcaccatcgacaccatcaccaccctcgaccagccggacagccgggcagagcagctcaacgccgcgctgaaccacatgatcaaccgggcgtcctccacggtgcgcagccggatcgatagcagccgactggcggtcatgggccactccatgggcggcggcggcaccctgcgtctggcctcccagcgtcccgacctgaaggccgccatcccgctcaccccgtggcacctcaacaagaactggagcagcgtcaccgtgccgacgctgatcatcggggccgacctcgacacgatcgcgccggtcgccacgcacgcgaaaccgttctacaacagcctgccgagctccatcagcaaggtgtacgtggagctcgacaatgcgtcgcacttcgcgcccaacagcaacaacgcggcgatctccgtgtacaccatctcgtggatgaagctgtgggtggataacgacacgcgctactccaccttcgcctgcgagaacccgaacagcacccgcgtgtcggacttccgcaccgcgaactgcagc

SEQ ID NO: 32 - DNA, 780 bp, IsPETase-8*Chimera-11
  source 1..780: mol_type = other DNA
tccaacccgtaccagcgcggtcccaaccccacgcggagcgcgctcacggccgacgggccgttctcggtcagcgaggagaacgtctcccggttgagcgccagcggcttcggcggcggcaccatctactacccgcgggagaacaacacctacggtgcggtggcgatctcccccggctacaccggcactgaggcttccatcgcctggctgggcgagcgcatcgcctcccacggcttcgtcgtcatcaccatcgacaccatcaccaccctcgaccagccggacagccgggcagagcagctcaacgccgcgctgaaccacatgatcaaccgggcgtcctccacggtgcgcagccggatcgatagcagccgactggcggtcatgggccactccatgggcggcggcggcaccctgcgtctggcctcccagcgtcccgacctgaaggccgccatcccgctcaccccgtggcacctcaacaagaactggagcagcgtcaccgtgccgacgctgatcatcggggccgacctcgacacgatcgcgccggtcgccacgcacgcgaaaccgttctacaacagcctgccgagctccatcagcaaggtgtacgtggagctcgacaatgcgtcgcacttcgcgcccaacagcaacaacgcggcgatctccgtgtacaccatctcgtggatgaagctgtgggtggataacgacacccgctacacccagttcctctgccccggaccgcgcgacggactcttcggcgaggtcgaagagtaccgctccacctgcccgttc

SEQ ID NO: 33 - DNA, 786 bp, IsPETase-8*Chimera-12
  source 1..786: mol_type = other DNA
gccaacccctacgagcgcggccccaacccgaccgacgccctgctcgaagccagcagcggccccttctccgtggcaacctacaccgtttcgcggctctcggtgagcggcttcgggggcggggtgatctactaccccacaggcacctcgctgaccttcggcgggatcgccatgtcgccggggtacacggccgacgccagttcgctggcgtggctcgggcggcggttggcatcgcacggcttcgtcgtcatcaccatcgacaccatcaccaccctcgaccagccggacagccgggcagagcagctcaacgccgcgctgaaccacatgatcaaccgggcgtcctccacggtgcgcagccggatcgatagcagccgactggcggtcatgggccactccatgggcggcggcggcaccctgcgtctggcctcccagcgtcccgacctgaaggccgccatcccgctcaccccgtggcacctcaacaagaactggagcagcgtcaccgtgccgacgctgatcatcggggccgacctcgacacgatcgcgccggtcgccacgcacgcgaaaccgttctacaacagcctgccgagctccatcagcaaggtgtacgtggagctcgacaatgcgtcgcacttcgcgcccaacagcaacaacgcggcgatctccgtgtacaccatctcgtggatgaagctgtgggtggataacgacacccgctacacccagttcctctgccccggaccgcgcgacggactcttcggcgaggtcgaagagtaccgctccacctgcccgttc

SEQ ID NO: 34 - DNA, 780 bp, IsPETase-8*Chimera-13
  source 1..780: mol_type = other DNA
tccaacccgtaccagcgcggtcccaaccccacgcggagcgcgctcacggccgacgggccgttctcggtggcaacctacaccgtttcgcggctctcggtgagcggcttcgggggcggggtgatctactaccccacaggcacctcgctgaccttcggtgcggtggcgatctcccccggctacaccggcactgaggcttccatcgcctggctgggcgagcgcatcgcctcccacggcttcgtcgtcatcaccatcgacaccatcaccaccctcgaccagccggacagccgggcagagcagctcaacgccgcgctgaaccacatgatcaaccgggcgtcctccacggtgcgcagccggatcgatagcagccgactggcggtcatgggccactcgatgggcggcggcgggaccctccgcatcgcagagcagaacccgtcgctgaaagcggccgtaccgctcacgccgtggcacaccgacaagacgttcaacacgtcggtaccggtgctgatcatcggggccgacctcgacacgatcgcgccggtcgccacgcacgcgaaaccgttctacaacagcctgccgagctccatcagcaaggtgtacgtggagctcgacaatgcgtcgcacttcgcgcccaacagcaacaacgcggcgatctccgtgtacaccatctcgtggatgaagctgtgggtggataacgacacccgctacacccagttcctctgccccggaccgcgcgacggactcttcggcgaggtcgaagagtaccgctccacctgcccgttc

SEQ ID NO: 35 - DNA, 780 bp, IsPETase-8*Chimera-14
  source 1..780: mol_type = other DNA
gccaacccctacgagcgcggccccaacccgaccgacgccctgctcgaagccagcagcggccccttctccgtcagcgaggagaacgtctcccggttgagcgccagcggcttcggcggcggcaccatctactacccgcgggagaacaacacctacggtgcggtggcgatctcccccggctacaccggcactgaggcttccatcgcctggctgggcgagcgcatcgcctcccacggcttcgtcgtcatcaccatcgacaccatcaccaccctcgaccagccggacagccgggcagagcagctcaacgccgcgctgaaccacatgatcaaccgggcgtcctccacggtgcgcagccggatcgatagcagccgactggcggtcatgggccactcgatgggcggcggcgggaccctccgcatcgcagagcagaacccgtcgctgaaagcggccgtaccgctcacgccgtggcacaccgacaagacgttcaacacgtcggtaccggtgctgatcatcggggccgacctcgacacgatcgcgccggtcgccacgcacgcgaaaccgttctacaacagcctgccgagctccatcagcaaggtgtacgtggagctcgacaatgcgtcgcacttcgcgcccaacagcaacaacgcggcgatctccgtgtacaccatctcgtggatgaagctgtgggtggataacgacacccgctacacccagttcctctgccccggaccgcgcgacggactcttcggcgaggtcgaagagtaccgctccacctgcccgttc

SEQ ID NO: 36 - DNA, 783 bp, IsPETase-8*Chimera-15
  source 1..783: mol_type = other DNA
gccaacccctacgagcgcggccccaacccgaccgacgccctgctcgaagccagcagcggccccttctccgtggcaacctacaccgtttcgcggctctcggtgagcggcttcgggggcggggtgatctactaccccacaggcacctcgctgaccttcggtgcggtggcgatctcccccggctacaccggcactgaggcttccatcgcctggctgggcgagcgcatcgcctcccacggcttcgtcgtcatcaccatcgacaccatcaccaccctcgaccagccggacagccgggcagagcagctcaacgccgcgctgaaccacatgatcaaccgggcgtcctccacggtgcgcagccggatcgatagcagccgactggcggtcatgggccactccatgggcggcggcggcaccctgcgtctggcctcccagcgtcccgacctgaaggccgccatcccgctcaccccgtggcacctcaacaagaactggagcagcgtcaccgtgccgacgctgatcttcgcctgcgagaacgacagcatcgccccggtcaactcgtccgccctgccgatctacgacagcatgtcgcgcaatgcgaaggtgtacgtggagctcgacaatgcgtcgcacttcgcgcccaacagcaacaacgcggcgatctccgtgtacaccatctcgtggatgaagctgtgggtggataacgacacccgctacacccagttcctctgccccggaccgcgcgacggactcttcggcgaggtcgaagagtaccgctccacctgcccgttc

SEQ ID NO: 37 - DNA, 789 bp, IsPETase-8*Chimera-16
  source 1..789: mol_type = other DNA
cagaccaacccctacgcccgcggcccgaacccgacagccgcctcactcgaagccagcgccggcccgttcaccgtggcaacctacaccgtttcgcggctctcggtgagcggcttcgggggcggggtgatctactaccccacaggcacctcgctgaccttcggtgcggtggcgatctcccccggctacaccggcactgaggcttccatcgcctggctgggcgagcgcatcgcctcccacggcttcgtcgtcatcaccatcgacaccatcaccaccctcgaccagccggacagccgggcagagcagctcaacgccgcgctgaaccacatgatcaaccgggcgtcctccacggtgcgcagccggatcgatagcagccgactggcggtcatgggccactccatgggcggcggcggcaccctgcgtctggcctcccagcgtcccgacctgaaggccgccatcccgctcaccccgtggcacctcaacaagaactggagcagcgtcaccgtgccgacgctgatcatcggggccgacctcgacacgatcgcgccggtcgccacgcacgcgaaaccgttctacaacagcctgccgagctccatcagcaaggtgtacgtggagctcgacaatgcgtcgcacttcgcgcccaacagcaacaacgcggcgatctccgtgtacaccatctcgtggatgaagctgtgggtggataacgacacccgctacacccagttcctctgccccggaccgcgcgacggactcttcggcgaggtcgaagagtaccgctccacctgcccgttc

SEQ ID NO: 38 - DNA, 783 bp, IsPETase-8*Chimera-17
  source 1..783: mol_type = other DNA
tccaacccgtaccagcgcggtcccaaccccacgcggagcgcgctcacggccgacgggccgttctcggtggcaacctacaccgtttcgcggctctcggtgagcggcttcgggggcggggtgatctactaccccacaggcacctcgctgaccttcggtgcggtggcgatctcccccggctacaccggcactgaggcttccatcgcctggctgggcgagcgcatcgcctcccacggcttcgtcgtcatcaccatcgacaccatcaccaccctcgaccagccggacagccgggcagagcagctcaacgccgcgctgaaccacatgatcaaccgggcgtcctccacggtgcgcagccggatcgatagcagccgactggcggtcatgggccactccatgggcggcggcggcaccctgcgtctggcctcccagcgtcccgacctgaaggccgccatcccgctcaccccgtggcacctcaacaagaactggagcagcgtcaccgtgccgacgctgatcatcggggccgacctcgacacgatcgcgccggtcgccacgcacgcgaaaccgttctacaacagcctgccgagctccatcagcaaggtgtacgtggagctcgacaatgcgtcgcacttcgcgcccaacagcaacaacgcggcgatctccgtgtacaccatctcgtggatgaagctgtgggtggataacgacacccgctacacccagttcctctgccccggaccgcgcgacggactcttcggcgaggtcgaagagtaccgctccacctgcccgttc

SEQ ID NO: 39 - DNA, 783 bp, IsPETase-8*Chimera-18
  source 1..783: mol_type = other DNA
gccaacccctacgagcgcggccccaacccgaccgacgccctgctcgaagccagcagcggccccttctccgtcagcgaggagaacgtctcccggttgagcgccagcggcttcggcggcggcaccatctactacccgcgggagaacaacacctacggtgcggtggcgatctcccccggctacaccggcactgaggcttccatcgcctggctgggcgagcgcatcgcctcccacggcttcgtcgtcatcaccatcgacaccatcaccaccctcgaccagccggacagccgggcagagcagctcaacgccgcgctgaaccacatgatcaaccgggcgtcctccacggtgcgcagccggatcgatagcagccgactggcggtcatgggccactccatgggcggcggcggcaccctgcgtctggcctcccagcgtcccgacctgaaggccgccatcccgctcaccccgtggcacctcaacaagaactggagcagcgtcaccgtgccgacgctgatcatcggggccgacctcgacacgatcgcgccggtcgccacgcacgcgaaaccgttctacaacagcctgccgagctccatcagcaaggtgtacgtggagctcgacaatgcgtcgcacttcgcgcccaacagcaacaacgcggcgatctccgtgtacaccatctcgtggatgaagctgtgggtggataacgacacccgctacacccagttcctctgccccggaccgcgcgacggactcttcggcgaggtcgaagagtaccgctccacctgcccgttc

SEQ ID NO: 40 - DNA, 783 bp, IsPETase-8*Chimera-19
  source 1..783: mol_type = other DNA
gccaacccctacgagcgcggccccaacccgaccgacgccctgctcgaagccagcagcggccccttctccgtggcaacctacaccgtttcgcggctctcggtgagcggcttcgggggcggggtgatctactaccccacaggcacctcgctgaccttcggtgcggtggcgatctcccccggctacaccggcactgaggcttccatcgcctggctgggcgagcgcatcgcctcccacggcttcgtcgtcatcaccatcgacaccatcaccaccctcgaccagccggacagccgggcagagcagctcaacgccgcgctgaaccacatgatcaaccgggcgtcctccacggtgcgcagccggatcgatagcagccgactggcggtcatgggccactcgatgggcggcggcgggaccctccgcatcgcagagcagaacccgtcgctgaaagcggccgtaccgctcacgccgtggcacaccgacaagacgttcaacacgtcggtaccggtgctgatcatcggggccgacctcgacacgatcgcgccggtcgccacgcacgcgaaaccgttctacaacagcctgccgagctccatcagcaaggtgtacgtggagctcgacaatgcgtcgcacttcgcgcccaacagcaacaacgcggcgatctccgtgtacaccatctcgtggatgaagctgtgggtggataacgacacccgctacacccagttcctctgccccggaccgcgcgacggactcttcggcgaggtcgaagagtaccgctccacctgcccgttc

SEQ ID NO: 41 - DNA, 786 bp, IsPETase-8*Chimera-20
  source 1..786: mol_type = other DNA
gccaacccctacgagcgcggccccaacccgaccgacgccctgctcgaagccagcagcggccccttctccgtggcaacctacaccgtttcgcggctctcggtgagcggcttcgggggcggggtgatctactaccccacaggcacctcgctgaccttcggtgcggtggcgatctcccccggctacaccggcactgaggcttccatcgcctggctgggcgagcgcatcgcctcccacggcttcgtcgtcatcaccatcgacaccatcaccaccctcgaccagccggacagccgggcagagcagctcaacgccgcgctgaaccacatgatcaaccgggcgtcctccacggtgcgcagccggatcgatagcagccgactggcggtcatgggccactccatgggcggcggcggcaccctgcgtctggcctcccagcgtcccgacctgaaggccgccatcccgctcaccccgtggcacctcaacaagaactggagcagcgtcaccgtgccgacgctgatcatcggggccgacctcgacacgatcgcgccggtcgccacgcacgcgaaaccgttctacaacagcctgccgagctccatcagcaaggtgtacgtggagctcgacaatgcgtcgcacttcgcgcccaacagcaacaacgcggcgatctccgtgtacaccatctcgtggatgaagctgtgggtggataacgacacccgctacacccagttcctctgccccggaccgcgcgacggactcttcggcgaggtcgaagagtaccgctccacctgcccgttc

SEQ ID NO: 42 - DNA, 867 bp, PET-IsPETase
  source 1..867: mol_type = genomic DNA
aactttccccgcgcttcccgcctgatgcaggccgccgttctcggcgggctgatggccgtgtcggccgccgccaccgcccagaccaacccctacgcccgcggcccgaacccgacagccgcctcactcgaagccagcgccggcccgttcaccgtgcgctcgttcaccgtgagccgcccgagcggctacggcgccggcaccgtgtactaccccaccaacgccggcggcaccgtgggcgccatcgccatcgtgccgggctacaccgcgcgccagtcgagcatcaaatggtggggcccgcgcctggcctcgcacggcttcgtggtcatcaccatcgacaccaactccacgctcgaccagccgtccagccgctcgtcgcagcagatggccgcgctgcgccaggtggcctcgctcaacggcaccagcagcagcccgatctacggcaaggtcgacaccgcccgcatgggcgtgatgggctggtcgatgggcggtggcggctcgctgatctcggcggccaacaacccgtcgctgaaagccgcggcgccgcaggccccgtgggacagctcgaccaacttctcgtcggtcaccgtgcccacgctgatcttcgcctgcgagaacgacagcatcgccccggtcaactcgtccgccctgccgatctacgacagcatgtcgcgcaatgcgaagcagttcctcgaaatcaacggtggctcgcactcctgcgccaacagcggcaacagcaaccaggcgctgatcggcaagaagggcgtggcctggatgaagcgcttcatggacaacgacacgcgctactccaccttcgcctgcgagaacccgaacagcacccgcgtgtcggacttccgcaccgcgaactgcagc

SEQ ID NO: 43 - DNA, 903 bp, PET-TfCUT2
  source 1..903: mol_type = genomic DNA
atggctgtgatgaccccccgccgggagcgctcttccctgctctcccgagctctgcaagtgacggctgcggctgccacagcgcttgtgaccgcggtcagcctggccgcccccgctcatgccgccaacccctacgagcgcggccccaacccgaccgacgccctgctcgaagccagcagcggccccttctccgtcagcgaggagaacgtctcccggttgagcgccagcggcttcggcggcggcaccatctactacccgcgggagaacaacacctacggtgcggtggcgatctcccccggctacaccggcactgaggcttccatcgcctggctgggcgagcgcatcgcctcccacggcttcgtcgtcatcaccatcgacaccatcaccaccctcgaccagccggacagccgggcagagcagctcaacgccgcgctgaaccacatgatcaaccgggcgtcctccacggtgcgcagccggatcgatagcagccgactggcggtcatgggccactccatgggcggcggcggcaccctgcgtctggcctcccagcgtcccgacctgaaggccgccatcccgctcaccccgtggcacctcaacaagaactggagcagcgtcaccgtgccgacgctgatcatcggggccgacctcgacacgatcgcgccggtcgccacgcacgcgaaaccgttctacaacagcctgccgagctccatcagcaaggcctacctggagctggacggcgcaacccacttcgccccgaacatccccaacaagatcatcggcaagtacagcgtcgcctggctcaagcggttcgtcgacaacgacacccgctacacccagttcctctgccccggaccgcgcgacggactcttcggcgaggtcgaagagtaccgctccacctgcccgttc

SEQ ID NO: 44 - DNA, 879 bp, PET-LCC
  source 1..879: mol_type = genomic DNA
atggacggagttctctggcgagtgcgaaccgcggcgctcatggccgcgctgctcgccctcgcagcctgggcgctggtctgggcttcgcccagcgtcgaggctcaatccaacccgtaccagcgcggtcccaaccccacgcggagcgcgctcacggccgacgggccgttctcggtggcaacctacaccgtttcgcggctctcggtgagcggcttcgggggcggggtgatctactaccccacaggcacctcgctgaccttcggcgggatcgccatgtcgccggggtacacggccgacgccagttcgctggcgtggctcgggcggcggttggcatcgcacggcttcgtggtgctcgtcatcaacacgaactcgcgattcgactaccctgactcccgcgcaagccagctatcggcggcgctgaactacctgcggacgagcagcccctcagccgtacgcgcccggctcgatgcgaaccgcctggccgttgcggggcattcgatgggcggcggcgggaccctccgcatcgcagagcagaacccgtcgctgaaagcggccgtaccgctcacgccgtggcacaccgacaagacgttcaacacgtcggtaccggtgctcatcgtgggagcggaagcggacacggtcgcgcccgtgagccagcacgccattccgttctaccagaacttgccctcgaccacgccgaaggtgtacgtggagctcgacaatgcgtcgcacttcgcgcccaacagcaacaacgcggcgatctccgtgtacaccatctcgtggatgaagctgtgggtggataacgacacccgctaccggcagttcctctgcaacgtgaacgatccggcgctgagcgacttccggacgaacaaccgccactgccag

SEQ ID NO: 45 - DNA, 45 bp, IsPETase-cSP-F
  source 1..45: mol_type = other DNA
gagatatacatatgcagaccaacccctacgcccgcggcccgaacc

SEQ ID NO: 46 - DNA, 45 bp, IsPETase-cSP-R
  source 1..45: mol_type = other DNA
gtaggggttggtctgcatatgtatatctccttcttaaagttaaac

SEQ ID NO: 47 - DNA, 45 bp, TfCut2-cSP-F
  source 1..45: mol_type = other DNA
ggagatatacatatggccaacccctacgagcgcggccccaacccg

SEQ ID NO: 48 - DNA, 45 bp, TfCut2-cSP-R
  source 1..45: mol_type = other DNA
ctcgtaggggttggccatatgtatatctccttcttaaagttaaac

SEQ ID NO: 49 - DNA, 45 bp, LCC-cSP-F
  source 1..45: mol_type = other DNA
ggagatatacatatggacggagttctctggcgagtgcgaaccgcg

SEQ ID NO: 50 - DNA, 45 bp, LCC-cSP-R
  source 1..45: mol_type = other DNA
ccagagaactccgtccatatgtatatctccttcttaaagttaaac

SEQ ID NO: 51 - DNA, 789 bp, pET-22b-IsPETase-cSP
  source 1..789: mol_type = other DNA
cagaccaacccctacgcccgcggcccgaacccgacagccgcctcactcgaagccagcgccggcccgttcaccgtgcgctcgttcaccgtgagccgcccgagcggctacggcgccggcaccgtgtactaccccaccaacgccggcggcaccgtgggcgccatcgccatcgtgccgggctacaccgcgcgccagtcgagcatcaaatggtggggcccgcgcctggcctcgcacggcttcgtggtcatcaccatcgacaccaactccacgctcgaccagccgtccagccgctcgtcgcagcagatggccgcgctgcgccaggtggcctcgctcaacggcaccagcagcagcccgatctacggcaaggtcgacaccgcccgcatgggcgtgatgggctggtcgatgggcggtggcggctcgctgatctcggcggccaacaacccgtcgctgaaagccgcggcgccgcaggccccgtgggacagctcgaccaacttctcgtcggtcaccgtgcccacgctgatcttcgcctgcgagaacgacagcatcgccccggtcaactcgtccgccctgccgatctacgacagcatgtcgcgcaatgcgaagcagttcctcgaaatcaacggtggctcgcactcctgcgccaacagcggcaacagcaaccaggcgctgatcggcaagaagggcgtggcctggatgaagcgcttcatggacaacgacacgcgctactccaccttcgcctgcgagaacccgaacagcacccgcgtgtcggacttccgcaccgcgaactgcagc

SEQ ID NO: 52 - protein, 263 aa, pET-22b-IsPETase-cSP
QTNPYARGPNPTAASLEASAGPFTVRSFTVSRPSGYGAGTVYYPTNAGGTVGAIAIVPGYTARQSSIKWWGPRLASHGFVVITIDTNSTLDQPSSRSSQQMAALRQVASLNGTSSSPIYGKVDTARMGVMGWSMGGGGSLISAANNPSLKAAAPQAPWDSSTNFSSVTVPTLIFACENDSIAPVNSSALPIYDSMSRNAKQFLEINGGSHSCANSGNSNQALIGKKGVAWMKRFMDNDTRYSTFACENPNSTRVSDFRTANCS

SEQ ID NO: 53 - DNA, 783 bp, pET-22b-TfCut2-cSP
  source 1..783: mol_type = other DNA
gccaacccctacgagcgcggccccaacccgaccgacgccctgctcgaagccagcagcggccccttctccgtcagcgaggagaacgtctcccggttgagcgccagcggcttcggcggcggcaccatctactacccgcgggagaacaacacctacggtgcggtggcgatctcccccggctacaccggcactgaggcttccatcgcctggctgggcgagcgcatcgcctcccacggcttcgtcgtcatcaccatcgacaccatcaccaccctcgaccagccggacagccgggcagagcagctcaacgccgcgctgaaccacatgatcaaccgggcgtcctccacggtgcgcagccggatcgatagcagccgactggcggtcatgggccactccatgggcggcggcggcaccctgcgtctggcctcccagcgtcccgacctgaaggccgccatcccgctcaccccgtggcacctcaacaagaactggagcagcgtcaccgtgccgacgctgatcatcggggccgacctcgacacgatcgcgccggtcgccacgcacgcgaaaccgttctacaacagcctgccgagctccatcagcaaggcctacctggagctggacggcgcaacccacttcgccccgaacatccccaacaagatcatcggcaagtacagcgtcgcctggctcaagcggttcgtcgacaacgacacccgctacacccagttcctctgccccggaccgcgcgacggactcttcggcgaggtcgaagagtaccgctccacctgcccgttc

SEQ ID NO: 54 - protein, 261 aa, pET-22b-TfCut2-cSP
ANPYERGPNPTDALLEASSGPFSVSEENVSRLSASGFGGGTIYYPRENNTYGAVAISPGYTGTEASIAWLGERIASHGFVVITIDTITTLDQPDSRAEQLNAALNHMINRASSTVRSRIDSSRLAVMGHSMGGGGTLRLASQRPDLKAAIPLTPWHLNKNWSSVTVPTLIIGADLDTIAPVATHAKPFYNSLPSSISKAYLELDGATHFAPNIPNKIIGKYSVAWLKRFVDNDTRYTQFLCPGPRDGLFGEVEEYRSTCPF

SEQ ID NO: 55 - DNA, 774 bp, pET-22b-LCC-cSP
  source 1..774: mol_type = other DNA
tccaacccgtaccagcgcggtcccaaccccacgcggagcgcgctcacggccgacgggccgttctcggtggcaacctacaccgtttcgcggctctcggtgagcggcttcgggggcggggtgatctactaccccacaggcacctcgctgaccttcggcgggatcgccatgtcgccggggtacacggccgacgccagttcgctggcgtggctcgggcggcggttggcatcgcacggcttcgtggtgctcgtcatcaacacgaactcgcgattcgactaccctgactcccgcgcaagccagctatcggcggcgctgaactacctgcggacgagcagcccctcagccgtacgcgcccggctcgatgcgaaccgcctggccgttgcggggcattcgatgggcggcggcgggaccctccgcatcgcagagcagaacccgtcgctgaaagcggccgtaccgctcacgccgtggcacaccgacaagacgttcaacacgtcggtaccggtgctcatcgtgggagcggaagcggacacggtcgcgcccgtgagccagcacgccattccgttctaccagaacttgccctcgaccacgccgaaggtgtacgtggagctcgacaatgcgtcgcacttcgcgcccaacagcaacaacgcggcgatctccgtgtacaccatctcgtggatgaagctgtgggtggataacgacacccgctaccggcagttcctctgcaacgtgaacgatccggcgctgagcgacttccggacgaacaaccgccactgccag

SEQ ID NO: 56 - protein, 258 aa, pET-22b-LCC-cSP
SNPYQRGPNPTRSALTADGPFSVATYTVSRLSVSGFGGGVIYYPTGTSLTFGGIAMSPGYTADASSLAWLGRRLASHGFVVLVINTNSRFDYPDSRASQLSAALNYLRTSSPSAVRARLDANRLAVAGHSMGGGGTLRIAEQNPSLKAAVPLTPWHTDKTFNTSVPVLIVGAEADTVAPVSQHAIPFYQNLPSTTPKVYVELDNASHFAPNSNNAAISVYTISWMKLWVDNDTRYRQFLCNVNDPALSDFRTNNRHCQ

SEQ ID NO: 57 - DNA, 45 bp, 8*chimera18-1-F
  source 1..45: mol_type = other DNA
gaagctgtgggtggataacgacacccgctacacccagttcctctg

SEQ ID NO: 58 - DNA, 35 bp, 8*chimera18-1-R
  source 1..35: mol_type = other DNA
gctccacgtacaccttgctgatggagctcggcagg

SEQ ID NO: 59 - DNA, 36 bp, 8*chimera18-2-F
  source 1..36: mol_type = other DNA
ccgagctccatcagcaaggtgtacgtggagctcgac

SEQ ID NO: 60 - DNA, 45 bp, 8*chimera18-2-R
  source 1..45: mol_type = other DNA
cagaggaactgggtgtagcgggtgtcgttatccacccacagcttc